European Patent Application EP 4 516 315 A1, published March 5, 2025. Title: ANTI-HUMAN IL-4RA ANTIBODY AND APPLICATION THEREOF. Applicant: Akeso Biopharma, Inc. The sequence listing filed with the application follows.

SEQUENCE LISTING (71 sequences)

SEQ ID NO: 1 - DNA, 348 bp, synthetic construct
  source 1..348: mol_type = other DNA
gaggtgcagctgcagcagagcggaccagagctggtgaagcctggcgcctctgtgaagatcagctgtaagacctccggctacaccttcacagagtatacaatccactgggtgaagcagaaccacggcaagagcctggagtggatcggcggcatcaatcctaacaatggcggcaccgtgtacaaccagaacttcaagggcaaggccaccctgacagtggacaagagctcctctaccgcctatatggagctgaggtctctgacaagcgaggactccgccgtgtactattgcgccagagtgcggagaggcatggattactggggccagggcacctccgtgacagtgagctcc

SEQ ID NO: 2 - protein, 116 aa, synthetic construct
EVQLQQSGPELVKPGASVKISCKTSGYTFTEYTIHWVKQNHGKSLEWIGGINPNNGGTVYNQNFKGKATLTVDKSSSTAYMELRSLTSEDSAVYYCARVRRGMDYWGQGTSVTVSS

SEQ ID NO: 3 - DNA, 321 bp, synthetic construct
  source 1..321: mol_type = other DNA
gacatcgtgatgacccagtcccacaagtttatgtccacatctgtgggcgacagggtgtccatcacctgtaaggcctctcaggatgtgaccacagccgtggcctggtaccagcagaagccaggccagtctcccaagctgctgatctatagcgcctcctaccggtatacaggcgtgcccgacagattcaccggctctggcagcggcacagatttcacctttacaatcagctccgtgcaggcagaggacctggccgtgtactattgccagcagcactactctgccccttggaccttcggcggaggaacaaacctggagatcaag

SEQ ID NO: 4 - protein, 107 aa, synthetic construct
DIVMTQSHKFMSTSVGDRVSITCKASQDVTTAVAWYQQKPGQSPKLLIYSASYRYTGVPDRFTGSGSGTDFTFTISSVQAEDLAVYYCQQHYSAPWTFGGGTNLEIK

SEQ ID NO: 5 - protein, 8 aa, synthetic construct
GYTFTEYT

SEQ ID NO: 6 - protein, 8 aa, synthetic construct
INPNNGGT

SEQ ID NO: 7 - protein, 9 aa, synthetic construct
ARVRRGMDY

SEQ ID NO: 8 - protein, 6 aa, synthetic construct
QDVTTA

SEQ ID NO: 9 - skipped

SEQ ID NO: 10 - protein, 9 aa, synthetic construct
QQHYSAPWT

SEQ ID NO: 11 - DNA, 348 bp, synthetic construct
  source 1..348: mol_type = other DNA
caggtgcagctgcagcagtccggagcagaggtggtgaagccaggagccagcgtgaagatctcctgtaagacctctggctacaccttcacagagtatacaatccactgggtgaagcaggcacacggacagagcctggagtggatcggcggcatcaaccctaacaatggcggcaccgtgtacaatcagaagtttcagggcaaggccaccctgacagtggacaagtctaccagcacagcctatatggagctgaggtccctgacctctgaggacacagccgtgtactattgcgcccgggtgcggagaggcatggattactggggccagggcacctccgtgacagtgagctcc

SEQ ID NO: 12 - protein, 116 aa, synthetic construct
QVQLQQSGAEVVKPGASVKISCKTSGYTFTEYTIHWVKQAHGQSLEWIGGINPNNGGTVYNQKFQGKATLTVDKSTSTAYMELRSLTSEDTAVYYCARVRRGMDYWGQGTSVTVSS

SEQ ID NO: 13 - DNA, 321 bp, synthetic construct
  source 1..321: mol_type = other DNA
gacatccagatgacccagtctcctaagtctctgagcacatccgtgggcgaccgggtgaccatcacatgtagagccagccaggatgtgaccacagcagtggcatggtaccagcagaagcctggcaagtcccctaagctgctgatctattctgccagctacaggtataccggagtgccatctcggttctccggctctggcagcggcacagacttcacctttacaatcagctccgtgcagccagaggatctggccacctactattgccagcagcactacagcgccccatggacctttggcggaggaacaaacctggagatcaag

SEQ ID NO: 14 - protein, 107 aa, synthetic construct
DIQMTQSPKSLSTSVGDRVTITCRASQDVTTAVAWYQQKPGKSPKLLIYSASYRYTGVPSRFSGSGSGTDFTFTISSVQPEDLATYYCQQHYSAPWTFGGGTNLEIK

SEQ ID NO: 15 - DNA, 348 bp, synthetic construct
  source 1..348: mol_type = other DNA
caggtgcagctggtgcagtccggagcagaggtggtgaagccaggagccagcgtgaaggtgtcctgtaagacctctggctacaccttcacagagtatacaatccactgggtgcggcaggcaccaggacagtctctggagtggatcggcggcatcaaccctaacaatggcggcaccaactacaatcagaagtttcagggcaaggtgaccctgacagtggacaagtccacctctacagcctatatggagctgagctccctgaggtctgaggacacagccgtgtactattgcgcccgcgtgcggagaggcatggattactggggccagggcaccagcgtgacagtgtctagc

SEQ ID NO: 16 - protein, 116 aa, synthetic construct
QVQLVQSGAEVVKPGASVKVSCKTSGYTFTEYTIHWVRQAPGQSLEWIGGINPNNGGTNYNQKFQGKVTLTVDKSTSTAYMELSSLRSEDTAVYYCARVRRGMDYWGQGTSVTVSS

SEQ ID NO: 17 - DNA, 321 bp, synthetic construct
  source 1..321: mol_type = other DNA
gacatccagatgacccagagccctagctccctgagcgcctccgtgggcgacagggtgaccatcacatgtagagcctcccaggatgtgaccacagcagtggcatggtaccagcagaagccaggcaaggcccctaagctgctgatctactccgcctctagcaggtataccggagtgccatctcggttctctggcagcggctccggcacagactttaccctgacaatctcctctgtgcagccagaggatctggccacatactattgccagcagcactattctgccccctggacctttggcggcggcacaaacctggagatcaag

SEQ ID NO: 18 - protein, 107 aa, synthetic construct
DIQMTQSPSSLSASVGDRVTITCRASQDVTTAVAWYQQKPGKAPKLLIYSASSRYTGVPSRFSGSGSGTDFTLTISSVQPEDLATYYCQQHYSAPWTFGGGTNLEIK

SEQ ID NO: 19 - DNA, 348 bp, synthetic construct
  source 1..348: mol_type = other DNA
caggtgcagctggtgcagtccggagcagaggtggtgaagccaggagccagcgtgaaggtgtcctgtaaggcctctggctacaccttcacagagtataccatccactgggtgcggcaggcaccaggacagggactggagtggatcggcggcatcaaccctaacaatggcggcacaaattacgcccagaagtttcagggcagggtgaccatcacagtggacaagtccacctctacagcctatatggagctgagctccctgaggtctgaggacaccgccgtgtactattgcgcccgcgtgcggagaggcatggattactggggccagggcaccagcgtgacagtgtctagc

SEQ ID NO: 20 - protein, 116 aa, synthetic construct
QVQLVQSGAEVVKPGASVKVSCKASGYTFTEYTIHWVRQAPGQGLEWIGGINPNNGGTNYAQKFQGRVTITVDKSTSTAYMELSSLRSEDTAVYYCARVRRGMDYWGQGTSVTVSS

SEQ ID NO: 21 - DNA, 321 bp, synthetic construct
  source 1..321: mol_type = other DNA
gacatccagatgacccagagccctagctccctgagcgcctccgtgggcgacagggtgaccatcacatgtagagcctcccaggatgtgaccacagccctggcatggtaccagcagaagccaggcaaggcccctaagctgctgatctactccgcctctagcctgtataccggagtgccatctcggttctctggcagcggctccggcacagactttaccctgacaatctcctctctgcagccagaggatttcgccacatactattgccagcagcactattctgccccctggacctttggcggcggcacaaacctggagatcaag

SEQ ID NO: 22 - protein, 107 aa, synthetic construct
DIQMTQSPSSLSASVGDRVTITCRASQDVTTALAWYQQKPGKAPKLLIYSASSLYTGVPSRFSGSGSGTDFTLTISSLQPEDFATYYCQQHYSAPWTFGGGTNLEIK

SEQ ID NO: 23 - DNA, 348 bp, synthetic construct
  source 1..348: mol_type = other DNA
caggtgcagctggtgcagtccggagcagaggtggtgaagccaggagccagcgtgaaggtgtcctgtaagacctctggctacaccttcacagagtatacaatccactgggtgcggcaggcaccaggacagtctctggagtggatcggcggcatcaaccctaacaatggcggcaccgtctacaatcagaagtttcagggcaaggtgaccctgacagtggacaagtccacctctacagcctatatggagctgagctccctgaggtctgaggacacagccgtgtactattgcgcccgcgtgcggagaggcatggattactggggccagggcaccagcgtgacagtgtctagc

SEQ ID NO: 24 - protein, 116 aa, synthetic construct
QVQLVQSGAEVVKPGASVKVSCKTSGYTFTEYTIHWVRQAPGQSLEWIGGINPNNGGTVYNQKFQGKVTLTVDKSTSTAYMELSSLRSEDTAVYYCARVRRGMDYWGQGTSVTVSS

SEQ ID NO: 25 - DNA, 321 bp, synthetic construct
  source 1..321: mol_type = other DNA
gacatccagatgacccagagccctagctccctgagcgcctccgtgggcgacagggtgaccatcacatgtagagcctcccaggatgtgaccacagcagtggcatggtaccagcagaagccaggcaaggcccctaagctgctgatctactccgcctcttacaggtataccggagtgccatctcggttctctggcagcggctccggcacagactttaccctgacaatctcctctgtgcagccagaggatctggccacatactattgccagcagcactattctgccccctggacctttggcggcggcacaaacctggagatcaag

SEQ ID NO: 26 - protein, 107 aa, synthetic construct
DIQMTQSPSSLSASVGDRVTITCRASQDVTTAVAWYQQKPGKAPKLLIYSASYRYTGVPSRFSGSGSGTDFTLTISSVQPEDLATYYCQQHYSAPWTFGGGTNLEIK

SEQ ID NO: 27 - protein, 25 aa, synthetic construct
EVQLQQSGPELVKPGASVKISCKTS

SEQ ID NO: 28 - protein, 17 aa, synthetic construct
IHWVKQNHGKSLEWIGG

SEQ ID NO: 29 - protein, 38 aa, synthetic construct
VYNQNFKGKATLTVDKSSSTAYMELRSLTSEDSAVYYC

SEQ ID NO: 30 - protein, 11 aa, synthetic construct
WGQGTSVTVSS

SEQ ID NO: 31 - protein, 26 aa, synthetic construct
DIVMTQSHKFMSTSVGDRVSITCKAS

SEQ ID NO: 32 - protein, 17 aa, synthetic construct
VAWYQQKPGQSPKLLIY

SEQ ID NO: 33 - protein, 36 aa, synthetic construct
YRYTGVPDRFTGSGSGTDFTFTISSVQAEDLAVYYC

SEQ ID NO: 34 - protein, 10 aa, synthetic construct
FGGGTNLEIK

SEQ ID NO: 35 - protein, 25 aa, synthetic construct
QVQLQQSGAEVVKPGASVKISCKTS

SEQ ID NO: 36 - protein, 17 aa, synthetic construct
IHWVKQAHGQSLEWIGG

SEQ ID NO: 37 - protein, 38 aa, synthetic construct
VYNQKFQGKATLTVDKSTSTAYMELRSLTSEDTAVYYC

SEQ ID NO: 38 - protein, 11 aa, synthetic construct
WGQGTSVTVSS

SEQ ID NO: 39 - protein, 26 aa, synthetic construct
DIQMTQSPKSLSTSVGDRVTITCRAS

SEQ ID NO: 40 - protein, 17 aa, synthetic construct
VAWYQQKPGKSPKLLIY

SEQ ID NO: 41 - protein, 36 aa, synthetic construct
YRYTGVPSRFSGSGSGTDFTFTISSVQPEDLATYYC

SEQ ID NO: 42 - protein, 10 aa, synthetic construct
FGGGTNLEIK

SEQ ID NO: 43 - protein, 25 aa, synthetic construct
QVQLVQSGAEVVKPGASVKVSCKTS

SEQ ID NO: 44 - protein, 17 aa, synthetic construct
IHWVRQAPGQSLEWIGG

SEQ ID NO: 45 - protein, 38 aa, synthetic construct
NYNQKFQGKVTLTVDKSTSTAYMELSSLRSEDTAVYYC

SEQ ID NO: 46 - protein, 11 aa, synthetic construct
WGQGTSVTVSS

SEQ ID NO: 47 - protein, 26 aa, synthetic construct [sequence omitted]

SEQ ID NO: 48 - protein, 17 aa, synthetic construct
VAWYQQKPGKAPKLLIY

SEQ ID NO: 49 - protein, 36 aa, synthetic construct
SRYTGVPSRFSGSGSGTDFTLTISSVQPEDLATYYC

SEQ ID NO: 50 - protein, 10 aa, synthetic construct
FGGGTNLEIK

SEQ ID NO: 51 - protein, 25 aa, synthetic construct
QVQLVQSGAEVVKPGASVKVSCKAS

SEQ ID NO: 52 - protein, 17 aa, synthetic construct
IHWVRQAPGQGLEWIGG

SEQ ID NO: 53 - protein, 38 aa, synthetic construct
NYAQKFQGRVTITVDKSTSTAYMELSSLRSEDTAVYYC

SEQ ID NO: 54 - protein, 11 aa, synthetic construct
WGQGTSVTVSS

SEQ ID NO: 55 - protein, 26 aa, synthetic construct [sequence omitted]

SEQ ID NO: 56 - protein, 17 aa, synthetic construct
LAWYQQKPGKAPKLLIY

SEQ ID NO: 57 - protein, 36 aa, synthetic construct
SLYTGVPSRFSGSGSGTDFTLTISSLQPEDFATYYC

SEQ ID NO: 58 - protein, 10 aa, synthetic construct
FGGGTNLEIK

SEQ ID NO: 59 - protein, 25 aa, synthetic construct
QVQLVQSGAEVVKPGASVKVSCKTS

SEQ ID NO: 60 - protein, 17 aa, synthetic construct
IHWVRQAPGQSLEWIGG

SEQ ID NO: 61 - protein, 38 aa, synthetic construct
VYNQKFQGKVTLTVDKSTSTAYMELSSLRSEDTAVYYC

SEQ ID NO: 62 - protein, 11 aa, synthetic construct
WGQGTSVTVSS

SEQ ID NO: 63 - protein, 26 aa, synthetic construct [sequence omitted]

SEQ ID NO: 64 - protein, 17 aa, synthetic construct
VAWYQQKPGKAPKLLIY

SEQ ID NO: 65 - protein, 36 aa, synthetic construct
YRYTGVPSRFSGSGSGTDFTLTISSVQPEDLATYYC

SEQ ID NO: 66 - protein, 10 aa, synthetic construct
FGGGTNLEIK

SEQ ID NO: 67 - protein, 232 aa, synthetic construct
PRGPTIKPCPPCKCPAPNLLGGPSVFIFPPKIKDVLMISLSPIVTCVVVDVSEDDPDVQISWFVNNVEVHTAQTQTHREDYNSTLRVVSALPIQHQDWMSGKEFKCKVNNKDLPAPIERTISKPKGSVRAPQVYVLPPPEEEMTKKQVTLTCMVTDFMPEDIYVEWTNNGKTELNYKNTEPVLDSDGSYFMYSKLRVEKKNWVERNSYSCSVVHEGLHNHHTTKSFSRTPGK

SEQ ID NO: 68 - protein, 443 aa, synthetic construct
EVQLEQSGAELMKPGASVKISCKATGYTFTTYWIEWIKQRPGHSLEWIGEILPGSDSTYYNEKVKGKVTFTADASSNTAYMQLSSLTSEDSAVYYCARGDGFYVYWGQGTTLTVSSASTKGPSVFPLAPCSRSTSESTAALGCLVKDYFPEPVTVSWNSGALTSGVHTFPAVLQSSGLYSLSSVVTVPSSSLGTKTYTCNVDHKPSNTKVDKRVESKYGPPCPPCPAPEFLGGPSVFLFPPKPKDTLMISRTPEVTCVVVDVSQEDPEVQFNWYVDGVEVHNAKTKPREEQFNSTYRVVSVLTVLHQDWLNGKEYKCKVSNKGLPSSIEKTISKAKGQPREPQVYTLPPSQEEMTKNQVSLTCLVKGFYPSDIAVEWESNGQPENNYKTTPPVLDSDGSFFLYSRLTVDKSRWQEGNVFSCSVMHEALHNHYTQKSLSLSLGK

SEQ ID NO: 69 - protein, 214 aa, synthetic construct
DIELTQSPATLSVTPGDSVSLSCRASQSISNNLHWYQQKSHESPRLLIKYTSQSMSGIPSRFSGSGSGTDFTLSINSVETEDFGVYFCQQSGSWPRTFGGGTKLDIKRTVAAPSVFIFPPSDEQLKSGTASVVCLLNNFYPREAKVQWKVDNALQSGNSQESVTEQDSKDSTYSLSSTLTLSKADYEKHKVYACEVTHQGLSSPVTKSFNRGEC

SEQ ID NO: 70 - protein, 118 aa, synthetic construct
EVQLVESGGGLVQPGRSLRLSCEASGFTFDDYAMHWVRQAPGKGLEWVSGLSRTSVSIGYADSVKGRFTISRDNAKNSLYLEMNSLRPEDTALYYCAKWGTRGYFDYWGQGTLVTVSS

SEQ ID NO: 71 - protein, 107 aa, synthetic construct
DIQMTQSPSSVSASVGDRVTITCRASQDISIWLAWYQQSPGKAPKLLINVASRLQSGVPSRFSGSGSGTDFTLTINSLQPEDFVTYYCQQANSFPITFGQGTRLATK